European Patent Specification EP 3 322 718 B1, published October 4, 2023. Title: HISTONE ANTI-CANCER VACCINES. Applicant: Ruprecht-Karls-Universität Heidelberg Deutsches Krebsforschungszentrum Stiftung des öffentlichen Rechts. The sequence listing filed with the application follows.

SEQUENCE LISTING (13 sequences)

SEQ ID NO: 1 - protein, 66 aa, Homo sapiens
ARTKQTARKSTGGKAPRKQLATKAARKSAPSTGGVKKPHRYRPGTVALREIRRYQKSTELLIRKLP

SEQ ID NO: 2 - protein, 66 aa, Homo sapiens
ARTKQTARKSTGGKAPRKQLATKAARMSAPSTGGVKKPHRYRPGTVALREIRRYQKSTELLIRKLP

SEQ ID NO: 3 - protein, 10 aa, Homo sapiens
KQLATKAARM

SEQ ID NO: 4 - protein, 10 aa, Homo sapiens
QLATKAARMS

SEQ ID NO: 5 - protein, 10 aa, Homo sapiens
LATKAARMSA

SEQ ID NO: 6 - protein, 10 aa, Homo sapiens
ATKAARMSAP

SEQ ID NO: 7 - protein, 10 aa, Homo sapiens
TKAARMSAPS

SEQ ID NO: 8 - protein, 10 aa, Homo sapiens
KAARMSAPST

SEQ ID NO: 9 - protein, 10 aa, Homo sapiens
AARMSAPSTG

SEQ ID NO: 10 - protein, 10 aa, Homo sapiens
ARMSAPSTGG

SEQ ID NO: 11 - protein, 10 aa, Homo sapiens
RMSAPSTGGV

SEQ ID NO: 12 - protein, 10 aa, Homo sapiens
MSAPSTGGVK

SEQ ID NO: 13 - protein, 27 aa, Homo sapiens
KAPRKQLATKAARMSAPSTGGVKKPHR